European Patent Specification EP 3 502 254 B1, published November 6, 2024. Title: NOVEL STRUCTURALLY DESIGNED SHRNAS. Applicant: Cold Spring Harbor Laboratory Hannon, Gregory J. Cheloufi, Sihem. The sequence listing filed with the application follows.

SEQUENCE LISTING (36 sequences)

SEQ ID NO: 1 - RNA, 40 nt, Artificial
  pre-let-7c-miR-451 mimic hairpin
ugagguaguagguuguaugguuguacaaccuacuaccuca

SEQ ID NO: 2 - RNA, 67 nt, Mus musculus
ugagguaguagguuguaugguuuagaguuacacccugggaguuaacuguacaaccuucuagcuuucc

SEQ ID NO: 3 - RNA, 63 nt, Artificial
  p53 hairpin in the mir-30 backbone
cccacuacaaguacauguguaauagugaagccacagauguauuacacauguacuuguagugga

SEQ ID NO: 4 - RNA, 40 nt, Artificial
  p53 hairpin mimicking the miR-451 fold
uuacacauguacuuguaguggacuacaaguacauguguaa

SEQ ID NO: 5 - RNA, 41 nt, Mus musculus
aaaccguuaccauuacugaguuuaguaaugguaacgguucu

SEQ ID NO: 6 - RNA, 22 nt, Mus musculus
uccacuacaaguacauguguaa

SEQ ID NO: 7 - RNA, 61 nt, Artificial
  mir-30 based pre-1224-shp53
cacuacaaguacauguguaauagugaagccacagauguauuacacauguacuuguagugga

SEQ ID NO: 8 - RNA, 66 nt, Mus musculus
ggcugggauaucaucauauacuguaaguuugugaugagacacuacaguauagaugauguacuaguc

SEQ ID NO: 9 - RNA, 72 nt, Mus musculus
cuugggaauggcgaggaaaccguuaccauuacugaguuuaguaaugguaacgguucucuugcugcucccaca

SEQ ID NO: 10 - DNA, 462 bp, Artificial
  Fragment of the mir-144-451 cluster sequence comprising 5' and 3' miR-451 flanking sequences with engineered restriction sites
agatctgagcagggagcaggaagctgtgtgtgtccagccctgacctgtcctgttctgcccccagcccctcacagtgcttttcaagccatgcttcctgtgcccccagtggggccctggctgggatatcatcatatactgtaagtttgcgatgagacactacagtatagatgatgtactagtccgggcacccccagctctggagcctgacaaggaggacaggagagatgctgcaagcccaagaagctctctgctcagcctgtcacaacctactgactgccagggcacttgggaatggcaaggaaaccgttaccattactgagtttagtaatggtaatggttctcttgctatacccagaaaacgtgccaggaagagaactcaggaccctgaagcagactactggaagggagactccagctcaaacaaggcaggggtgggggcgtgggattgggggtaggacgcgt

SEQ ID NO: 11 - DNA, 41 bp, Mus musculus
aaaccgttaccattactgagtttagtaatggtaatggttct

SEQ ID NO: 12 - RNA, 23 nt, Homo sapiens
uaaggugcaucuagugcaguuag

SEQ ID NO: 13 - RNA, 21 nt, Homo sapiens
uaaggugcaucuagugcaguu

SEQ ID NO: 14 - RNA, 22 nt, Homo sapiens
uaaggugcaucuagugcaguua

SEQ ID NO: 15 - RNA, 23 nt, Homo sapiens
uaaggugcaucuagugcaguuag

SEQ ID NO: 16 - RNA, 22 nt, Homo sapiens
aaggugcaucuagugcaguuag

SEQ ID NO: 17 - RNA, 21 nt, Homo sapiens
aggugcaucuagugcaguuag

SEQ ID NO: 18 - RNA, 22 nt, Homo sapiens
uagcuuaucagacugauguuga

SEQ ID NO: 19 - RNA, 21 nt, Homo sapiens
uagcuuaucagacugauguug

SEQ ID NO: 20 - RNA, 22 nt, Homo sapiens
uagcuuaucagacugauguuga

SEQ ID NO: 21 - RNA, 21 nt, Homo sapiens
agcuuaucagacugauguuga

SEQ ID NO: 22 - DNA, 21 bp, Artificial
  Primer for genotyping Ago2 insertional alleles in Ago2-null mouse cells.
gacggtgaagaagcacaggaa

SEQ ID NO: 23 - DNA, 21 bp, Artificial
  Primer for genotyping Ago2 insertional alleles in Ago2-null mouse cells.
ggtccgatgggaaagtgtagc

SEQ ID NO: 24 - DNA, 18 bp, Artificial
  Primer for genotyping Ago2 insertional alleles in Ago2-null mouse cells.
atgggatcggccattgaa

SEQ ID NO: 25 - DNA, 18 bp, Artificial
  Primer for genotyping Ago2 insertional alleles in Ago2-null mouse cells.
gaactcgtcaagaaggcg

SEQ ID NO: 26 - DNA, 20 bp, Artificial
  RT-PCT primer for Ago2 insertional alleles in mice.
tgttccagcaacctgtcatc

SEQ ID NO: 27 - DNA, 20 bp, Artificial
  RT-PCT primer for Ago2 insertional alleles in mice.
gatgatctcctgtcggtgct

SEQ ID NO: 28 - DNA, 18 bp, Artificial
  RT-PCT primer for actin in mice.
atgctccccgggctgtat

SEQ ID NO: 29 - DNA, 24 bp, Artificial
  RT-PCR primer for actin in mice.
cataggagtccttctgacccattc

SEQ ID NO: 30 - DNA, 22 bp, Artificial
  Target Sequence for Renilla-shRNA-1
taggaattataatgcttatcta

SEQ ID NO: 31 - DNA, 22 bp, Artificial
  Reverse complement of Renilla-shRNA-1 Sequence
tagataagcattataattccta

SEQ ID NO: 32 - DNA, 18 bp, Artificial
  Trimmed reverse complement of Renilla-shRNA-1 target sequence
tagataagcattataatt

SEQ ID NO: 33 - DNA, 18 bp, Artificial
  Reverse complement of trimmed reverse complement of Renilla-shRNA-1 target sequence
aattataatgcttatcta

SEQ ID NO: 34 - DNA, 40 bp, Artificial
  Renilla-shRNA-1 sequence
tagataagcattataattcctaaattataatgcttatcta

SEQ ID NO: 35 - DNA, 40 bp, Artificial
  Renilla-shRNA-1 sequence with sequence substitution
tagataagcattataattcctaaattataatgcttatctc

SEQ ID NO: 36 - DNA, 164 bp, Artificial
  Renilla-shRNA-1 Sequence with miR451 flanking sequences
gaagctctctgctcagcctgtcacaacctactgactgccagggcacttgggaatggcaaggtagataagcattataattcctaaattataatgcttatctctcttgctatacccagaaaacgtgccaggaagagaactcaggaccctgaagcagactactggaa